European Patent Specification EP 3 369 420 B1, published March 12, 2025. Title: COMPOSITIONS AND METHODS FOR IMPROVING MITOCHONDRIAL FUNCTION AND TREATING NEURODEGENERATIVE DISEASES AND COGNITIVE DISORDERS. Applicant: Amazentis SA. The sequence listing filed with the application follows.

SEQUENCE LISTING (18 sequences)

SEQ ID NO: 1 - DNA, 23 bp, Artificial sequence
  Synthetic oligonucleotide
aagtgtggaactctctggaactg

SEQ ID NO: 2 - DNA, 23 bp, Artificial sequence
  Synthetic oligonucleotide
gggttatcttggttggctttatg

SEQ ID NO: 3 - DNA, 20 bp, Artificial sequence
  Synthetic oligonucleotide
aagtgtttttccagcatggg

SEQ ID NO: 4 - DNA, 20 bp, Artificial sequence
  Synthetic oligonucleotide
ggctgcaattttcctaacca

SEQ ID NO: 5 - DNA, 17 bp, Artificial sequence
  Synthetic oligonucleotide
tcatggaatagagcgcc

SEQ ID NO: 6 - DNA, 20 bp, Artificial sequence
  Synthetic oligonucleotide
gtgtgctcaccgattctaca

SEQ ID NO: 7 - DNA, 20 bp, Artificial sequence
  Synthetic oligonucleotide
cccatgtgctcctaccagat

SEQ ID NO: 8 - DNA, 20 bp, Artificial sequence
  Synthetic oligonucleotide
ccttgaagaagcgacctttg

SEQ ID NO: 9 - DNA, 26 bp, Artificial sequence
  Synthetic oligonucleotide
gatcgcaatgggtgcttttgatagaa

SEQ ID NO: 10 - DNA, 26 bp, Artificial sequence
  Synthetic oligonucleotide
agctgattggcaatgtctccagcaaa

SEQ ID NO: 11 - DNA, 24 bp, Artificial sequence
  Synthetic oligonucleotide
gtagcttatgaatgtgtgcaactc

SEQ ID NO: 12 - DNA, 24 bp, Artificial sequence
  Synthetic oligonucleotide
gtcttgcgatcagctctttcatta

SEQ ID NO: 13 - DNA, 20 bp, Artificial sequence
  Synthetic oligonucleotide
gcacacatttccccacactg

SEQ ID NO: 14 - DNA, 20 bp, Artificial sequence
  Synthetic oligonucleotide
cccaacctgcccattctgat

SEQ ID NO: 15 - DNA, 20 bp, Artificial sequence
  Synthetic oligonucleotide
tccatcagggtatcctctcc

SEQ ID NO: 16 - DNA, 20 bp, Artificial sequence
  Synthetic oligonucleotide
ggaggcaagcataagactgg

SEQ ID NO: 17 - DNA, 21 bp, Artificial sequence
  Synthetic oligonucleotide
acgtcaaagggtacctgtcca

SEQ ID NO: 18 - DNA, 21 bp, Artificial sequence
  Synthetic oligonucleotide
caatcccagatggcagaactt